European Patent Specification EP 3 674 704 B1, published May 3, 2023. Title: Method of isolation of exosome and Kit for isolation of exosome. Applicant: Hiroshima University. The sequence listing filed with the application follows.

SEQUENCE LISTING (7 sequences)

SEQ ID NO: 1 - protein, 4 aa, Artificial Sequence
  Artificially Synthesized Peptide Linker
GGGS

SEQ ID NO: 2 - protein, 5 aa, Artificial Sequence
  Artificially Synthesized Peptide Linker
GGGGS

SEQ ID NO: 3 - protein, 8 aa, Artificial Sequence
  Artificially Synthesized Peptide Linker
GGGSGGGS

SEQ ID NO: 4 - protein, 12 aa, Artificial Sequence
  Artificially Synthesized Peptide Linker
GGGSGGGSGGGS

SEQ ID NO: 5 - protein, 16 aa, Artificial Sequence
  Artificially Synthesized Sequence
GGGSGGGSGGGSKKKK

SEQ ID NO: 6 - protein, 20 aa, Artificial Sequence
  Artificially Synthesized Sequence
GGGSGGGSGGGSKKKKKKKK

SEQ ID NO: 7 - protein, 24 aa, Artificial Sequence
  Artificially Synthesized Sequence
GGGSGGGSKKKKKKKKKKKKKKKK